European Patent Application EP 4 286 537 A1, published December 6, 2023. Title: METHOD AND KIT FOR IDENTIFYING BACTERIUM CAUSING SEPTICEMIA. Applicant: Denka Company Limited Toho University. The sequence listing filed with the application follows.

SEQUENCE LISTING (163 sequences)

SEQ ID NO: 1 - DNA, 22 bp, Artificial Sequence
  Forward Primer(A.spp_3923F21)
cagcattgccagaataactttc

SEQ ID NO: 2 - DNA, 25 bp, Artificial Sequence
  Reverse Primer(A.spp_4056R25Y)
gatycgtaagaattttggtaaattg

SEQ ID NO: 3 - DNA, 23 bp, Artificial Sequence
  Forward Primer(A.bau_373F23)
tgatctgacgaagacacattaac

SEQ ID NO: 4 - DNA, 22 bp, Artificial Sequence
  Reverse Primer(A.bau_552R22)
atttcagtttagagcactgtgc

SEQ ID NO: 5 - DNA, 17 bp, Artificial Sequence
  Forward Primer(C. spp_449F17)
gctgcttcttcctgctg

SEQ ID NO: 6 - DNA, 18 bp, Artificial Sequence
  Forward Primer(C. spp_443F18S)
cagcttsttcctgctgac

SEQ ID NO: 7 - DNA, 19 bp, Artificial Sequence
  Reverse Primer(C. spp_551R19)
gtctggaataccagtggac

SEQ ID NO: 8 - DNA, 17 bp, Artificial Sequence
  Forward Primer(Enb.spp_216F17)
ggccgaagaagaagtct

SEQ ID NO: 9 - DNA, 19 bp, Artificial Sequence
  Reverse Primer(Enb.spp_369R19)
gcggatgagacctaarttg

SEQ ID NO: 10 - DNA, 19 bp, Artificial Sequence
  Forward Primer(E.coli_468F19)
ggttaccggcgagactgaa

SEQ ID NO: 11 - DNA, 18 bp, Artificial Sequence
  Reverse Primer(E.coli_567R18)
gacaactcacgcagacgt

SEQ ID NO: 12 - DNA, 18 bp, Artificial Sequence
  Forward Primer(K.aer_2097F18)
gcgtcgtcttcgataagc

SEQ ID NO: 13 - DNA, 24 bp, Artificial Sequence
  Reverse Primer(K.aer_1941R25)
gaagtttgatattcgtgaaaacag

SEQ ID NO: 14 - DNA, 18 bp, Artificial Sequence
  Forward Primer(K.pne_1886F19)
ggtgaacaccctggtctc

SEQ ID NO: 15 - DNA, 20 bp, Artificial Sequence
  Reverse Primer(K.pne_2043R20)
gatattccggccccataatg

SEQ ID NO: 16 - DNA, 17 bp, Artificial Sequence
  Forward Primer(K.oxy_261F17)
ccatttcggctaccgtc

SEQ ID NO: 17 - DNA, 21 bp, Artificial Sequence
  Reverse Primer(K.oxy_423R21)
cgatgaaagatatcgccaaag

SEQ ID NO: 18 - DNA, 18 bp, Artificial Sequence
  Forward Primer(K.var_1886F18)
ggtgaacaccctggtttc

SEQ ID NO: 19 - DNA, 18 bp, Artificial Sequence
  Reverse Primer(K.var_2046R18)
cgatattccggccccatg

SEQ ID NO: 20 - DNA, 18 bp, Artificial Sequence
  Forward Primer(Pse.aer_430F18)
ggtaaagagcgtccggtc

SEQ ID NO: 21 - DNA, 19 bp, Artificial Sequence
  Reverse Primer(Pse.aer_489R19)
ttacttcttcagctcgacg

SEQ ID NO: 22 - DNA, 20 bp, Artificial Sequence
  Forward Primer(Pro.spp_2356F20Y)
caactcactayggtcgtgtg

SEQ ID NO: 23 - DNA, 22 bp, Artificial Sequence
  Reverse Primer(Pro.spp_2226R22)
catctgttacagcgttgttttc

SEQ ID NO: 24 - DNA, 17 bp, Artificial Sequence
  Forward Primer(Ser.mar_349F17Y)
ggcctgaacctcagyag

SEQ ID NO: 25 - DNA, 18 bp, Artificial Sequence
  Reverse Primer(Ser.mar_459R19)
ccgtagtcgtcgaggatg

SEQ ID NO: 26 - DNA, 23 bp, Artificial Sequence
  Forward Primer(Enc. fae_121F23)
agtccctcatctaaaaaccattg

SEQ ID NO: 27 - DNA, 24 bp, Artificial Sequence
  Forward Primer(Enc.spp_3566F24Y)
tcaatcaaattcggtaattcyaat

SEQ ID NO: 28 - DNA, 23 bp, Artificial Sequence
  Forward Primer(Enc.spp_3563F23Y)
cgatcaaattyggtaattccaac

SEQ ID NO: 29 - DNA, 18 bp, Artificial Sequence
  Reverse Primer(Enc.spp_3639R18R)
arcttggctggacacgta

SEQ ID NO: 30 - DNA, 25 bp, Artificial Sequence
  Forward Primer(L.spp_444F25)
atgaatatgaaaaaagcaactatcg

SEQ ID NO: 31 - DNA, 20 bp, Artificial Sequence
  Reverse Primer(L.spp_551R20W)
gcgataccccaaagwgtatc

SEQ ID NO: 32 - DNA, 21 bp, Artificial Sequence
  Forward Primer(Sta.aur_566F21W)
gtagcgaaawagaaaaacctc

SEQ ID NO: 33 - DNA, 24 bp, Artificial Sequence
  Reverse Primer(Sta.aur_656R24)
atacttattaagtgctggcatatg

SEQ ID NO: 34 - DNA, 25 bp, Artificial Sequence
  Forward Primer(Sta.sch_226F25Y)
ttcaacttcaattttyttagcattc

SEQ ID NO: 35 - DNA, 25 bp, Artificial Sequence
  Forward Primer(Sta.arg_226F25)
ttccacttctattttcttagcattc

SEQ ID NO: 36 - DNA, 22 bp, Artificial Sequence
  Reverse Primer(Sta.arg_319R22Y)
attaattgatacgccygaaacg

SEQ ID NO: 37 - DNA, 20 bp, Artificial Sequence
  Forward Primer(Sta.epi_409F20)
agttgagacaggaaatggtc

SEQ ID NO: 38 - DNA, 19 bp, Artificial Sequence
  Reverse Primer(Sta.epi_544R19)
aggagtggtccacttcttc

SEQ ID NO: 39 - DNA, 20 bp, Artificial Sequence
  Forward Primer(Sta.spp_595F20Y)
tacatyccaactccagaacg

SEQ ID NO: 40 - DNA, 20 bp, Artificial Sequence
  Reverse Primer(Sta.spp_697R20)
actttgatttgaccacgttc

SEQ ID NO: 41 - DNA, 20 bp, Artificial Sequence
  Forward Primer(Str.spp_rnpB F20)
atgaggaaagtccatgctag

SEQ ID NO: 42 - DNA, 18 bp, Artificial Sequence
  Reverse Primer(Str.spp_rnpB R18)
ttgggttgctagcttgag

SEQ ID NO: 43 - DNA, 21 bp, Artificial Sequence
  Forward Primer(Str.pneu_371F21)
cctttgatttcatcctgcttg

SEQ ID NO: 44 - DNA, 21 bp, Artificial Sequence
  Reverse Primer(Str.pneu_459R21)
cacaaaactcagctcaatcac

SEQ ID NO: 45 - DNA, 22 bp, Artificial Sequence
  Forward Primer(Str.pyo_1623F22)
gccacctatttatggtgttaag

SEQ ID NO: 46 - DNA, 23 bp, Artificial Sequence
  Reverse Primer(Str.pyo_1800R23)
aacgattttcaggatccatagta

SEQ ID NO: 47 - DNA, 182 bp, Artificial Sequence
  Partial sequence of Acinetobacter spp. rpoB gene
gatccgtaagaattttggtaaattgccccaagtaatggatgcaccgtacttattatcgattcaggtcgattcgtacagaacattcttgcaagatggcaaatcaccaaaaaaccgcgaagatatcggtctccaagccgcatttcgttcagtttttcctatcgaaagttattctggcaatgctg

SEQ ID NO: 48 - DNA, 198 bp, Artificial Sequence
  Partial sequence of Acinetobacter baumannii 16S-23S ITS gene
atttcagtttagagcactgtgcacttaagcaccgtacagcttcaatctaaattcacataccaaaacgcttgattcagttaatttgctagttctcaattcatctagattaattgcttaacctaaactcttgagtgaacaatttatttcagactcaattttgccaatctgttaatgagttaatgtgtcttcgtcagatca

SEQ ID NO: 49 - DNA, 118 bp, Artificial Sequence
  Partial sequence of Citrobacter spp. ompA gene
gtctggaataccagtggactaacaacatcggcgacgcaaacaccgttggcggtcgtccagataacggcctgctgagcgttggtgtttcctaccgtttcggccagcaggaagaagcagc

SEQ ID NO: 50 - DNA, 172 bp, Artificial Sequence
  Partial sequence of Enterobacter spp. rpoS gene
gcggatgagacctaagttgccctcttcaatcagatccagcagagccagaccacgattgccgtaacggcgggcaattttcacgaccagtcgcaggttactttcgatcatgcgacgacgcgaggcaacatcaccacgcaaagcacgacgtgcgaaatagacttcttcttcggcc

SEQ ID NO: 51 - DNA, 120 bp, Artificial Sequence
  Partial sequence of Escherichia coli gyrB gene
gacaactcacgcagacgtttcgccagaatttcatattcgaactcggtcacattggtgaaggtttcgaggctgggccagaaacgcaccatggtgccggttttttcagtctcgccggtaacc

SEQ ID NO: 52 - DNA, 174 bp, Artificial Sequence
  Partial sequence of Klebsiella aerogenes gyrB gene
gaagtttgatattcgtgaaaacagcgagctgcagcagttcgagcccatcgtgcgcgtgcgtacccacggcgtcgataccgactacccgttggataacgagttcatcaccggcgcggaatatcgccgcatctgcaccctcggcgagaagctgcgtgggcttatcgaagacgacgc

SEQ ID NO: 53 - DNA, 176 bp, Artificial Sequence
  Partial sequence of Klebsiella pneumoniae gyrB gene
gatattccggccccataatgaactcgttatccagcggatagtcggtatccacgccgtgggtacgtacgcgaataaccggctcaaaatgctgcagttctttgttctcgtggagatcgaatttccactggctgccgtgctgttctttctcgttcagctcggagaccagggtgttcacc

SEQ ID NO: 54 - DNA, 183 bp, Artificial Sequence
  Partial sequence of Klebsiella oxytoca pehX gene
cgatgaaagatatcgccaaagagccgttcgtttttactatcaaatacagcgccgacgtgaatgatacgacccctgccgacgagcccgctcagttccgcgacgttcaggtgcaggacgtcaccgtcgatggtacttcggctaagcacagcatcctgattgacggcatgacggtagccgaaatgg

SEQ ID NO: 55 - DNA, 177 bp, Artificial Sequence
  Partial sequence of Klebsiella variicola gyrB gene
cgatattccggccccatgatgaactcgttatccagcggatagtcggtatccaccccgtgggtacggacgcggataatcggctcaaactgctgcaattcaccgttctcgcggacatcaaatttccactggctgccgtgctgctctttctcattcagctcggaaaccagggtgttcacc

SEQ ID NO: 56 - DNA, 78 bp, Artificial Sequence
  Partial sequence of Pseudomonas aeruginosa oprL gene
ttacttcttcagctcgacgcgacggttctgagcccaggactgctcgtcgtggccggtagcgaccggacgctctttacc

SEQ ID NO: 57 - DNA, 150 bp, Artificial Sequence
  Partial sequence of Proteus spp. rpoB gene
catctgttacagcgttgttttctacaacacggtaaggcgtttctaagaatccgtactcgttagtctgtgcataaacagataatgagttaatcagaccgatatttggaccttcaggtgtttcgattggacacacacgaccatagtgagttg

SEQ ID NO: 58 - DNA, 128 bp, Artificial Sequence
  Partial sequence of Serratia marcescens hasA gene
ccgtagtcgtcgaggatgccgttcagcgcggtttccagcgcgccggtatcgccggacatcaggccgtacaccacctggtgcaccacgccatcgtggccctgcgcctgcaggctgctgaggttcaggcc

SEQ ID NO: 59 - DNA, 96 bp, Artificial Sequence
  Partial sequence of Enterococcus spp. rpoB gene
agcttggctggacacgtagtaaaatacggaaagcatcgcgaacgtagaagtttcgcacgtatcagtgaagtattggaattaccaaatttaattgaa

SEQ ID NO: 60 - DNA, 125 bp, Artificial Sequence
  Partial sequence of Listeria spp. iap p60 gene
gcgataccccaaagagtatcaccagcttcaactactacagtgcttgcggatgcgattgttggagcagcaaatgctgttaccgcaatcccagctgtagccgcgatagttgcttttttcatattcat

SEQ ID NO: 61 - DNA, 114 bp, Artificial Sequence
  Partial sequence of Staphylococcus aureus nuc gene
atacttattaagtgctggcatatgtatggcaattgtttcaatattacttatagggatggctatcagtaatgtttcgaaagaacaatacgcaaagaggtttttctttttcgctac

SEQ ID NO: 62 - DNA, 115 bp, Artificial Sequence
  Partial sequence of Staphylococcus argenteus nuc gene
attaattgatacgcctgaaacgaaacatcctaaaaaaggcgttgaaaaatatggcccagaagcaagtgcatttacgaagaatatggtagagaatgctaagaaaatagaagtggaa

SEQ ID NO: 63 - DNA, 151 bp, Artificial Sequence
  Partial sequence of Staphylococcus epidermidis atlE gene
aggagtggtccacttcttctgtttagcaaaactcttaccagtctttacagcatcttcatcaaaagcaccaataccaaaaaagttataatagtgatggttaccttctttaattccttttgataaatctgattgaccatttcctgtctcaact

SEQ ID NO: 64 - DNA, 122 bp, Artificial Sequence
  Partial sequence of Staphylococcus spp. tuf gene
actttgatttgaccacgttcaacacggcctgtagcaacagtaccacgaccagtgattgagaatacgtcctcaactggcatcatgaatggtttgtcagaatcacgttctggagttggaatgta

SEQ ID NO: 65 - DNA, 244 bp, Artificial Sequence
  Partial sequence of Streptococcus spp. rnpB gene
ttgggttgctagcttgaggggtttaccgcgttccactctctctgtttccagaaagacttcgtcactgtggcactttcaagcctactctggcctatccaaggacttagccatttcaactgccgtaacgatttctcgtccctaggcttatggtttcgcctagcacaaacactacaggcatcacagcctgtgctagcatggactttcctcatgagaagcaattctcctcacgcgattatccaaaaat

SEQ ID NO: 66 - DNA, 109 bp, Artificial Sequence
  Partial sequence of Streptococcus pneumoniae xisco gene
cacaaaactcagctcaatcacaagcttctaagcaattagctactgaaaaagaatcagctaaaaatgccattgaaaaagcagccaagaacaagcaggatgaaatcaaagg

SEQ ID NO: 67 - DNA, 200 bp, Artificial Sequence
  Partial sequence of Streptococcus pyogenes gyrB gene
aacgattttcaggatccatagtagtttcccaaagttgatggtcatccatttccccaagacctttataacgttgaacagttggttttgaacgaccaatactatatttttcaagagctgtttttaattggtcttcttgatcaatacctggctgaatgtactctttaatctcactaccgaccttaacaccataaataggtggc

SEQ ID NO: 68 - DNA, 20 bp, Artificial Sequence
  Forward Primer(KPC_167F20)
ctgtaagttaccgcgctgag

SEQ ID NO: 69 - DNA, 21 bp, Artificial Sequence
  Reverse Primer(KPC_376R21_B)
ggcgttatcactgtattgcac

SEQ ID NO: 70 - DNA, 19 bp, Artificial Sequence
  Forward Primer(NDM_178F19)
cagcacacttcctatctcg

SEQ ID NO: 71 - DNA, 20 bp, Artificial Sequence
  Reverse Primer(NDM_408R20)
cattggcataagtcgcaatc

SEQ ID NO: 72 - DNA, 22 bp, Artificial Sequence
  Forward Primer(IMP_307F22)
ggaatagrgtggcttaattctc

SEQ ID NO: 73 - DNA, 20 bp, Artificial Sequence
  Reverse Primer(IMP_478R20)
arccaaaccactacgttatc

SEQ ID NO: 74 - DNA, 18 bp, Artificial Sequence
  Forward Primer(VIM_155F18)
gtgtttggtcgcatatcg

SEQ ID NO: 75 - DNA, 18 bp, Artificial Sequence
  Reverse Primer(VIM_246R18)
ccccacgctgtatcaatc

SEQ ID NO: 76 - DNA, 20 bp, Artificial Sequence
  Forward Primer(CTX-M1_402F20)
taacgtggcgatgaataagc

SEQ ID NO: 77 - DNA, 20 bp, Artificial Sequence
  Reverse Primer(CTX-M1_631R20)
ttgcctttcatccaygtcac

SEQ ID NO: 78 - DNA, 20 bp, Artificial Sequence
  Forward Primer(CTX-M2_414F20)
gaayaagctgattgcccatc

SEQ ID NO: 79 - DNA, 18 bp, Artificial Sequence
  Reverse Primer(CTX-M2_633R18)
ttgcccttaagccacgtc

SEQ ID NO: 80 - DNA, 20 bp, Artificial Sequence
  Forward Primer(CTX-M2_414F20)
gaayaagctgattgcccatc

SEQ ID NO: 81 - DNA, 18 bp, Artificial Sequence
  Reverse Primer(CTX_M8_485R19)
gtgtyatccccaatcgca

SEQ ID NO: 82 - DNA, 20 bp, Artificial Sequence
  Forward Primer(CTX-M2_414F20)
gaayaagctgattgcccatc

SEQ ID NO: 83 - DNA, 20 bp, Artificial Sequence
  Reverse Primer(CTX_M25_485R21)
gtgtcatcgccaatcgtacg

SEQ ID NO: 84 - DNA, 17 bp, Artificial Sequence
  Forward Primer(CTX-M9_291F18)
tgtcgagatcaagcctg

SEQ ID NO: 85 - DNA, 20 bp, Artificial Sequence
  Reverse Primer(CTX-M9_411R20)
gggcaatcaatttgttcatg

SEQ ID NO: 86 - DNA, 18 bp, Artificial Sequence
  Forward Primer(OXA23_262F18)
atcggattggagaaccag

SEQ ID NO: 87 - DNA, 20 bp, Artificial Sequence
  Reverse Primer(OXA23_386R20)
cgcaagttcctgatagactg

SEQ ID NO: 88 - DNA, 22 bp, Artificial Sequence
  Forward Primer(OXA40_131F22
gctattttgatgaagctcaaac

SEQ ID NO: 89 - DNA, 21 bp, Artificial Sequence
  Reverse Primer(OXA40_232R22)
cttaaatgttgatgcagggac

SEQ ID NO: 90 - DNA, 21 bp, Artificial Sequence
  Forward Primer(OXA48_148F21)
aataagcagcaaggatttacc

SEQ ID NO: 91 - DNA, 19 bp, Artificial Sequence
  Reverse Primer(OXA48_252R19)
gtgttcatccttaaccacg

SEQ ID NO: 92 - DNA, 23 bp, Artificial Sequence
  Forward Primer(OXA58_516F23)
gcctttgacaattacacctatac

SEQ ID NO: 93 - DNA, 20 bp, Artificial Sequence
  Reverse Primer(OXA58_613R20)
cgctctacatacaacatctc

SEQ ID NO: 94 - DNA, 22 bp, Artificial Sequence
  Forward Primer(mecA_763F22)
gttatgttggtcccattaactc

SEQ ID NO: 95 - DNA, 20 bp, Artificial Sequence
  Reverse Primer(mecA_875R20)
gatagccatcttcatgttgg

SEQ ID NO: 96 - DNA, 18 bp, Artificial Sequence
  Forward Primer(vanA_808F18)
ggacggatacaggaaacg

SEQ ID NO: 97 - DNA, 22 bp, Artificial Sequence
  Reverse Primer(vanA_900R22)
attgacttcgttcagtacaatg

SEQ ID NO: 98 - DNA, 19 bp, Artificial Sequence
  Forward Primer(vanB_264F19)
gcgtattgatgtggctttc

SEQ ID NO: 99 - DNA, 20 bp, Artificial Sequence
  Reverse Primer(vanB_355R20)
ctttgaatatcacagcccac

SEQ ID NO: 100 - DNA, 230 bp, Artificial Sequence
  Partial sequence of Klebsiella pneumoniae Beta-Lactamase_KPC gene
ggcgttatcactgtattgcacggcggccgcggacagctccgccaccgtcatgcctgttgtcagatatttttccgagatgggtgaccacggaaccagcgcatttttgccgtaacggatgggtgtgtccagcaagccggcctgctgctggctgcgagccagcacagcggcagcaagaaagcccttgaatgagctgcacagtgggaagcgctcctcagcgcggtaacttacag

SEQ ID NO: 101 - DNA, 250 bp, Artificial Sequence
  Partial sequence of Klebsiella pneumoniae Beta-Lactamase_KDM gene
cattggcataagtcgcaatccccgccgcatgcagcgcgttcataccgcccatcttgtcctgatgcgcgtgagtcaccaccgccagcgcgaccggcaggttgatctcctgcttgatccagttgaggatctgggcggtctggtcatcggtccaggcggtatcgaccaccagcacgcggccgccatccctgacgatcaaaccgttggaagcgactgccccgaaacccggcatgtcgagataggaagtgtgctg

SEQ ID NO: 102 - DNA, 191 bp, Artificial Sequence
  Partial sequence of Pseudomonas aeruginosa Beta-Lactamase_IMP85 gene
agccaaaccactacgttatctggagtgtgccctggaccaggataaaaaacttcaatctttttcttaactagccaatagctagctccgctaaatgaatttttagcttgtactttaccgtcttttttaagaagttcatttgttaattcagatgcatacgtggggatagattgagaattaagccactctattcc

SEQ ID NO: 103 - DNA, 109 bp, Artificial Sequence
  Partial sequence of Citrobacter freundii Beta-Lactamase_VIM gene
ccccacgctgtatcaatcaaaagcaactcatcaccatcacggacaatgagaccattggacgggtagaccgcgccatcaaacgactgcgttgcgatatgcgaccaaacac

SEQ ID NO: 104 - DNA, 249 bp, Artificial Sequence
  Partial sequence of Salmonella enterica Beta-Lactamase_CTX-M1 gene
ttgcctttcatccatgtcaccagctgcgcccgttggctgtcacccaatgctttacccagcgtcagattacgcagagtttgcgccattgcccgaggtgaagtggtatcacgcggatcgcccggaatggcggtgtttaacgtcggctcggtacggtcgagacggaacgtttcgtctcccagctgtcgggcgaacgcggtgacgctagccgggccgccaacgtgagaaatcagcttattcatcgccacgtta

SEQ ID NO: 105 - DNA, 237 bp, Artificial Sequence
  Partial sequence of Salmonella enterica Beta-Lactamase_CTX-M2 gene
ttgcccttaagccacgtcaccaactgtgcccgctgagtttccgccagcgctttacccagcgtcagatttttcagggtctgcgccatcgcgagcggcgtggtggtatcacgcgggtcgcctggaatggcggtattgagcgtgggctcggttctgtccagacggaaggtctcatcacccaacgagcgagcaaacgccgtcactttatcgggaccacccagatgggcaatcagcttattc

SEQ ID NO: 106 - DNA, 72 bp, Artificial Sequence
  Partial sequence of Citrobacter amalonatics Beta-Lactamase_CTX-M8 gene
gtgttatccccaatcgcacgggcaaacgccgtcactttatccggccccccaagatgggcaatcagcttgttc

SEQ ID NO: 107 - DNA, 72 bp, Artificial Sequence
  Partial sequence of Escherichia coli Beta-Lactamase_CTX-M25 gene
gtgtcatcgccaatcgtacgggcaaatgccgtcactttatccggccccccgagatgggcaatcagcttattc

SEQ ID NO: 108 - DNA, 140 bp, Artificial Sequence
  Partial sequence of  Escherichia coli Beta-Lactamase_CTX-M9 gene
gggcaatcaatttgttcatggcggtattgtcgctgtactgcaacgcggccgcgctcagctctgccagcgtcattgtgccgttgacgtgtttttcggcaatcggattgtagttaaccagatcggcaggcttgatctcgaca

SEQ ID NO: 109 - DNA, 144 bp, Artificial Sequence
  Partial sequence of Acinetobacter baumannii Beta-Lactamase_OXA-23 gene
cgcaagttcctgatagactgggactgcagaaagcttcatggcttctcctagtgtcatgtctttttcccaagcggtaaatgaccttttctcgcccttccatttaaatatttcattaatatccgttttctggttctccaatccgat

SEQ ID NO: 110 - DNA, 122 bp, Artificial Sequence
  Partial sequence of Acinetobacter baumannii Beta-Lactamase_OXA-40 gene
cttaaatgttgatgcagggacatattctttatttgctcgtgcaagagcattaccataggtgctaagatttttaccctctttaataataattacaccctgtgtttgagcttcatcaaaatagc

SEQ ID NO: 111 - DNA, 123 bp, Artificial Sequence
  Partial sequence of Klebsiella pneumoniae Beta-Lactamase_OXA-48 gene
gtgttcatccttaaccacgcccaaatcgagggcgatcaagctattgggaattttaaaggtagatgcgggtaaaaatgcttggttcgcccgtttaagattattggtaaatccttgctgcttatt

SEQ ID NO: 112 - DNA, 117 bp, Artificial Sequence
  Partial sequence of Acinetobacter haemolyticus Beta-Lactamase_OXA-58 gene
cgctctacatacaacatctctttcacttgttgctgaacttcaggtttaaaaggcaattgcccttgggctaaatcatacacaaactttacttcttgtataggtgtaattgtcaaaggc

SEQ ID NO: 113 - DNA, 132 bp, Artificial Sequence
  Partial sequence of Staphylococcus aureus mecA gene
gatagccatcttcatgttggagctttttatcgtaaagtttttcgagtccctttttaccaataactgcatcatctttatagcctttatattctttttgttttaattcttcagagttaatgggaccaacataac

SEQ ID NO: 114 - DNA, 114 bp, Artificial Sequence
  Partial sequence of Enterococcus faecalis vanA gene
attgacttcgttcagtacaatgcggccgttatcttgtaaaaacatatccacacgggctagacctctacagccgagcgctttatatattttttttgccgtttcctgtatccgtcc

SEQ ID NO: 115 - DNA, 111 bp, Artificial Sequence
  Partial sequence of Enterococcus faecium vanB gene
ctttgaatatcacagcccacataggggataccagacaatacaaacagcccctgtatcgcaccatcctccccgcatttgccatgcaaaaccgggaaagccacatcaatacgc

SEQ ID NO: 116 - DNA, 25 bp, Artificial Sequence
  A.spp_P1 (rpoB)
ttttttttttttcgcggttttttgg

SEQ ID NO: 117 - DNA, 25 bp, Artificial Sequence
  A.spp_172P17
ttttttttataggaaaaactgaacg

SEQ ID NO: 118 - DNA, 25 bp, Artificial Sequence
  A.bau_P19
ttttttgaatttagattgaagctgt

SEQ ID NO: 119 - DNA, 25 bp, Artificial Sequence
  C. spp_24P17R
ttttttttgaaacggtargaaacac

SEQ ID NO: 120 - DNA, 25 bp, Artificial Sequence
  Enb.spp_349P17
ttttttttctggatctgattgaaga

SEQ ID NO: 121 - DNA, 25 bp, Artificial Sequence
  E.coli_531P16
tttttttttcaatgtgaccgagttc

SEQ ID NO: 122 - DNA, 25 bp, Artificial Sequence
  K.aer_2034P17
ttttttttggtgatgaactcgttat

SEQ ID NO: 123 - DNA, 25 bp, Artificial Sequence
  K.oxy_392P17R
ttttttttgcrctgtatttgatagt

SEQ ID NO: 124 - DNA, 25 bp, Artificial Sequence
  K.pne_P16
tttttttttgaactgcagcattttg

SEQ ID NO: 125 - DNA, 25 bp, Artificial Sequence
  K.var_1968P16
tttttttttgttgcagcagtttgag

SEQ ID NO: 126 - DNA, 25 bp, Artificial Sequence
  Pse.aer_430P15
ttttttttttggtaaagagcgtccg

SEQ ID NO: 127 - DNA, 25 bp, Artificial Sequence
  Pro.spp_P16
ttttttttttagaaacgccttaccg

SEQ ID NO: 128 - DNA, 25 bp, Artificial Sequence
  Ser.mar_424P14
tttttttttttatgtccggcgatac

SEQ ID NO: 129 - DNA, 25 bp, Artificial Sequence
  Enc.spp_3607P14
tttttttttttcttctacgttcgcg

SEQ ID NO: 130 - DNA, 25 bp, Artificial Sequence
  Enc.spp_3606P15
ttttttttttgcttctacgttctcg

SEQ ID NO: 131 - DNA, 25 bp, Artificial Sequence
  Enc.spp_Probe A
ttttttttgatgctttccgtatttt

SEQ ID NO: 132 - DNA, 25 bp, Artificial Sequence
  L.spp_533P16_1
tttttttttgtagtagtcgaagctg

SEQ ID NO: 133 - DNA, 25 bp, Artificial Sequence
  L.spp_533P17_2
ttttttttgtagtagttgaagctgg

SEQ ID NO: 134 - DNA, 25 bp, Artificial Sequence
  Sta.aur_625P21
ttttccctataagtaatattgaaac

SEQ ID NO: 135 - DNA, 25 bp, Artificial Sequence
  Sta.arg_288P17
ttttttttcatatttttcaacgcct

SEQ ID NO: 136 - DNA, 25 bp, Artificial Sequence
  Sta.epi_505P20
tttttgatgctgtaaagactggtaa

SEQ ID NO: 137 - DNA, 25 bp, Artificial Sequence
  Sta.spp_626P16
tttttttttaaccattcatgatgcc

SEQ ID NO: 138 - DNA, 25 bp, Artificial Sequence
  Str.pneu_440P17
ttttttttgctaattgcttagaagc

SEQ ID NO: 139 - DNA, 25 bp, Artificial Sequence
  Str.pyo_1783P17
ttttttttcatcaactttgggaaac

SEQ ID NO: 140 - DNA, 25 bp, Artificial Sequence
  Str.spp_Probe B
tttttttttttttgccacagtgacg

SEQ ID NO: 141 - DNA, 25 bp, Artificial Sequence
  NDM_365P16
tttttttttatcaggacaagatggg

SEQ ID NO: 142 - DNA, 25 bp, Artificial Sequence
  KPC_330P18
tttttttatatctgacaacaggcat

SEQ ID NO: 143 - DNA, 25 bp, Artificial Sequence
  VIM_232P17
ttttttttgatgagttgcttttgat

SEQ ID NO: 144 - DNA, 25 bp, Artificial Sequence
  IMP_378P16K
tttttttttagacggtaaggtkcaa

SEQ ID NO: 145 - DNA, 25 bp, Artificial Sequence
  OXA23_373P15
ttttttttttctttctgcagtccca

SEQ ID NO: 146 - DNA, 25 bp, Artificial Sequence
  OXA40_217P19
ttttttgcaaataaagaatatgtcc

SEQ ID NO: 147 - DNA, 25 bp, Artificial Sequence
  OXA48_223P16
tttttttttcccaatagcttgatcg

SEQ ID NO: 148 - DNA, 25 bp, Artificial Sequence
  OXA58_596P16
tttttttttttcagcaacaagtgaa

SEQ ID NO: 149 - DNA, 25 bp, Artificial Sequence
  CTX-M1_594P15
ttttttttttgggtaaagcattggg

SEQ ID NO: 150 - DNA, 25 bp, Artificial Sequence
  CTX-M2_465P14
ttttttttttttcgctcgttgggtg

SEQ ID NO: 151 - DNA, 25 bp, Artificial Sequence
  CTX-M8_485P20
tttttttataaagtgacggcgtttg

SEQ ID NO: 152 - DNA, 25 bp, Artificial Sequence
  CTX-M9_393P16
tttttttttgtacagcgacaatacc

SEQ ID NO: 153 - DNA, 25 bp, Artificial Sequence
  CTX-M25_485P20
tttttttataaagtgacggcatttg

SEQ ID NO: 154 - DNA, 25 bp, Artificial Sequence
  mecA_822P17
ttttttttgatgatgcagttattgg

SEQ ID NO: 155 - DNA, 25 bp, Artificial Sequence
  vanA_867P16
tttttttttccgtgtggatatgttt

SEQ ID NO: 156 - DNA, 25 bp, Artificial Sequence
  vanB_331P18
ttttttttttgtattgtctggtatc

SEQ ID NO: 157 - DNA, 17 bp, Artificial Sequence
  Forward Primer (E.coli_1969F17)
caaaacctgttcgagcc

SEQ ID NO: 158 - DNA, 18 bp, Artificial Sequence
  Reverse Primer (E.coli_2093R18)
cttcttccagcaagccac

SEQ ID NO: 159 - DNA, 25 bp, Artificial Sequence
  E.coli_526P15
ttttttttttttcaccaatgtgacc

SEQ ID NO: 160 - DNA, 18 bp, Artificial Sequence
  Forward Primer (C. spp_568F18)
tcygatagccagccgatg

SEQ ID NO: 161 - DNA, 18 bp, Artificial Sequence
  Reverse Primer (C. spp(3)_670R18)
cattgcgtgggtcagttt

SEQ ID NO: 162 - DNA, 25 bp, Artificial Sequence
  C. spp_55P15Y
ttttttttttccgttatcyggacga

SEQ ID NO: 163 - DNA, 25 bp, Artificial Sequence
  C. spp_65P19R
ttttttgacgaccrccaacggtgtt